European Patent Application EP 4 524 164 A1, published March 19, 2025. Title: 新融合蛋白及其用途. Applicant: 南京吉盛澳玛生物医药有限公司. The sequence listing filed with the application follows.

SEQUENCE LISTING (12 sequences)

SEQ ID NO: 1 - protein, 133 aa, synthetic construct [sequence omitted]

SEQ ID NO: 2 - protein, 133 aa, synthetic construct
APTSSSTKKTQLQLEHLLLDLQMILNGINNYKNPKLTAMLTFKFYMPKKATELKHLQCLEEELKPLEEVLNLAQSKNFHFDPRDVVSNINVFVLELKGSETTFMCEYADETATIVEFLNRWITFCQSIISTLT

SEQ ID NO: 3 - protein, 379 aa, synthetic construct
APTSSSTKKTQLQLEHLLLDLQMILNGINNYKNPKLTAMLTFKFYMPKKATELKHLQCLEEELKPLEEVLNLAQSKNFHFDPRDVVSNINVFVLELKGSETTFMCEYADETATIVEFLNRWITFCQSIISTLTGGGGSGGGGSGGGGSEPKSCDKTHTCPPCPAPEAAGGPSVFLFPPKPKDTLYITREPEVTCVVVDVSHEDPEVKFNWYVDGVEVHNAKTKPREEQYNSTYRVVSVLTVLHQDWLNGKEYKCKVSNKALPAPIEKTISKAKGQPREPQVYTLPPSREEMTKNQVSLTCLVKGFYPSDIAVEWESNGQPENNYKTTPPVLDSDGSFFLYSKLTVDKSRWQQGNVFSCSVMHEALHNHYTQKSLSLSPK

SEQ ID NO: 4 - protein, 379 aa, synthetic construct
EPKSCDKTHTCPPCPAPEAAGGPSVFLFPPKPKDTLYITREPEVTCVVVDVSHEDPEVKFNWYVDGVEVHNAKTKPREEQYNSTYRVVSVLTVLHQDWLNGKEYKCKVSNKALPAPIEKTISKAKGQPREPQVYTLPPSREEMTKNQVSLTCLVKGFYPSDIAVEWESNGQPENNYKTTPPVLDSDGSFFLYSKLTVDKSRWQQGNVFSCSVMHEALHNHYTQKSLSLSPAGGGGSGGGGSGGGGSAPTSSSTKKTQLQLEHLLLDLQMILNGINNYKNPKLTAMLTFKFYMPKKATELKHLQCLEEELKPLEEVLNLAQSKNFHFDPRDVVSNINVFVLELKGSETTFMCEYADETATIVEFLNRWITFCQSIISTLT

SEQ ID NO: 5 - protein, 165 aa, synthetic construct
CDLPQTHSLGSRRTLMLLAQMRRISLFSCLKDRHDFGFPQEEFGNQFQKAETIPVLHEMIQQIFNLFSTKDSSAAWDETLLDKFYTELYQQLNDLEACVIQGVGVTETPLMNEDSILAVRKYFQRITLYLKEKKYSPCAWEVVRAEIMRSFSLSTNLQESLRSKE

SEQ ID NO: 6 - protein, 165 aa, synthetic construct
CDLPQTHSLGSRRTLMLLAQMRRISLFSCLKDRHDFGFPQEEFGNQFQKAETIPVLHEMIQQIFNLFSTKDSSAAWDETLLDKFYTELYQQLNDLEACVIQGVGVTETPLMNEDSILAVRKYFQRITLYLKEKKYSPCAWEVVAAEIMRSFSLSTNLQESLRSKE

SEQ ID NO: 7 - protein, 411 aa, synthetic construct
CDLPQTHSLGSRRTLMLLAQMRRISLFSCLKDRHDFGFPQEEFGNQFQKAETIPVLHEMIQQIFNLFSTKDSSAAWDETLLDKFYTELYQQLNDLEACVIQGVGVTETPLMNEDSILAVRKYFQRITLYLKEKKYSPCAWEVVAAEIMRSFSLSTNLQESLRSKEGGGGSGGGGSGGGGSEPKSCDKTHTCPPCPAPEAAGGPSVFLFPPKPKDTLYITREPEVTCVVVDVSHEDPEVKFNWYVDGVEVHNAKTKPREEQYNSTYRVVSVLTVLHQDWLNGKEYKCKVSNKALPAPIEKTISKAKGQPREPQVYTLPPSREEMTKNQVSLTCLVKGFYPSDIAVEWESNGQPENNYKTTPPVLDSDGSFFLYSKLTVDKSRWQQGNVFSCSVMHEALHNHYTQKSLSLSPK

SEQ ID NO: 8 - protein, 411 aa, synthetic construct
EPKSCDKTHTCPPCPAPEAAGGPSVFLFPPKPKDTLYITREPEVTCVVVDVSHEDPEVKFNWYVDGVEVHNAKTKPREEQYNSTYRVVSVLTVLHQDWLNGKEYKCKVSNKALPAPIEKTISKAKGQPREPQVYTLPPSREEMTKNQVSLTCLVKGFYPSDIAVEWESNGQPENNYKTTPPVLDSDGSFFLYSKLTVDKSRWQQGNVFSCSVMHEALHNHYTQKSLSLSPAGGGGSGGGGSGGGGSCDLPQTHSLGSRRTLMLLAQMRRISLFSCLKDRHDFGFPQEEFGNQFQKAETIPVLHEMIQQIFNLFSTKDSSAAWDETLLDKFYTELYQQLNDLEACVIQGVGVTETPLMNEDSILAVRKYFQRITLYLKEKKYSPCAWEVVAAEIMRSFSLSTNLQESLRSKE

SEQ ID NO: 9 - protein, 559 aa, synthetic construct
APTSSSTKKTQLQLEHLLLDLQMILNGINNYKNPKLTAMLTFKFYMPKKATELKHLQCLEEELKPLEEVLNLAQSKNFHFDPRDVVSNINVFVLELKGSETTFMCEYADETATIVEFLNRWITFCQSIISTLTGGGGSGGGGSGGGGSEPKSCDKTHTCPPCPAPEAAGGPSVFLFPPKPKDTLYITREPEVTCVVVDVSHEDPEVKFNWYVDGVEVHNAKTKPREEQYNSTYRVVSVLTVLHQDWLNGKEYKCKVSNKALPAPIEKTISKAKGQPREPQVYTLPPSREEMTKNQVSLTCLVKGFYPSDIAVEWESNGQPENNYKTTPPVLDSDGSFFLYSKLTVDKSRWQQGNVFSCSVMHEALHNHYTQKSLSLSPAGGGGSGGGGSGGGGSCDLPQTHSLGSRRTLMLLAQMRRISLFSCLKDRHDFGFPQEEFGNQFQKAETIPVLHEMIQQIFNLFSTKDSSAAWDETLLDKFYTELYQQLNDLEACVIQGVGVTETPLMNEDSILAVRKYFQRITLYLKEKKYSPCAWEVVAAEIMRSFSLSTNLQESLRSKE

SEQ ID NO: 10 - protein, 559 aa, synthetic construct
CDLPQTHSLGSRRTLMLLAQMRRISLFSCLKDRHDFGFPQEEFGNQFQKAETIPVLHEMIQQIFNLFSTKDSSAAWDETLLDKFYTELYQQLNDLEACVIQGVGVTETPLMNEDSILAVRKYFQRITLYLKEKKYSPCAWEVVAAEIMRSFSLSTNLQESLRSKEGGGGSGGGGSGGGGSEPKSCDKTHTCPPCPAPEAAGGPSVFLFPPKPKDTLYITREPEVTCVVVDVSHEDPEVKFNWYVDGVEVHNAKTKPREEQYNSTYRVVSVLTVLHQDWLNGKEYKCKVSNKALPAPIEKTISKAKGQPREPQVYTLPPSREEMTKNQVSLTCLVKGFYPSDIAVEWESNGQPENNYKTTPPVLDSDGSFFLYSKLTVDKSRWQQGNVFSCSVMHEALHNHYTQKSLSLSPAGGGGSGGGGSGGGGSAPTSSSTKKTQLQLEHLLLDLQMILNGINNYKNPKLTAMLTFKFYMPKKATELKHLQCLEEELKPLEEVLNLAQSKNFHFDPRDVVSNINVFVLELKGSETTFMCEYADETATIVEFLNRWITFCQSIISTLT

SEQ ID NO: 11 - protein, 15 aa, synthetic construct
GGGGSGGGGSGGGGS

SEQ ID NO: 12 - protein, 231 aa, synthetic construct
EPKSCDKTHTCPPCPAPEAAGGPSVFLFPPKPKDTLYITREPEVTCVVVDVSHEDPEVKFNWYVDGVEVHNAKTKPREEQYNSTYRVVSVLTVLHQDWLNGKEYKCKVSNKALPAPIEKTISKAKGQPREPQVYTLPPSREEMTKNQVSLTCLVKGFYPSDIAVEWESNGQPENNYKTTPPVLDSDGSFFLYSKLTVDKSRWQQGNVFSCSVMHEALHNHYTQKSLSLSPK